European Patent Specification EP 3 708 574 B1, published January 24, 2024. Title: Peptide for Inhibiting Skin Inflammation And Composition for Preventing or Treating Skin Inflammation Containing The Same. Applicant: AVIXGEN Inc. The sequence listing filed with the application follows.

SEQUENCE LISTING (3 sequences)

SEQ ID NO: 1 - protein, 4 aa, Artificial Sequence
  tetrapeptide
RLYE

SEQ ID NO: 2 - protein, 39 aa, Artificial Sequence
  ACP
VKCFNCGKEGHTARNCRAPRKKGCWKCGKEGHQMKDCTE

SEQ ID NO: 3 - protein, 43 aa, Artificial Sequence
  ACP-tetrapeptide
VKCFNCGKEGHTARNCRAPRKKGCWKCGKEGHQMKDCTERLYE